European Patent Specification EP 3 508 574 B1, published October 9, 2024. Title: METHOD OF INTEGRATING DNA FRAGMENT OF INTEREST INTO REGION ADJACENT TO BINDING SITE OF DNA BINDING PROTEIN. Applicant: KYUSHU UNIVERSITY TOKYO INSTITUTE OF TECHNOLOGY. The sequence listing filed with the application follows.

SEQUENCE LISTING (4 sequences)

SEQ ID NO: 1 - DNA, 67 bp, Artificial Sequence
  A DNA fragment for ChILT method
atgcattaatacgactcactatagggtagatcgctcgtcggcagcgtcagatgtgtataagagacag

SEQ ID NO: 2 - DNA, 19 bp, Artificial Sequence
  A DNA fragment for ChILT method
ctgtctcttatacacatct

SEQ ID NO: 3 - DNA, 34 bp, Artificial Sequence
  A DNA fragment for ChILT method
gtctcgtgggctcggagatgtgtataagagacag

SEQ ID NO: 4 - DNA, 19 bp, Artificial Sequence
  A DNA fragment for ChILT method
ctgtctcttatacacatct